European Patent Application EP 4 647 436 A2, published November 12, 2025. Title: Biologically active cluster of molecules. Applicant: Sampreme Technologies B.V. Application EP. The sequence listing filed with the application follows.

SEQUENCE LISTING (10 sequences)

SEQ ID NO: 1 - DNA, 16 bp, synthetic construct
  source 1..16: mol_type = other DNA; note = Antisense BNA (HSP27) oligo nucleic acid sequence
ggcacagccagtggcg

SEQ ID NO: 2 - DNA, 18 bp, synthetic construct
  source 1..18: mol_type = other DNA; note = UBC primer forward sequence
cagccgggatttgggtcg

SEQ ID NO: 3 - DNA, 23 bp, synthetic construct
  source 1..23: mol_type = other DNA; note = UBC primer reverse sequence
cacgaagatctgcattgtcaagt

SEQ ID NO: 4 - DNA, 20 bp, synthetic construct
  source 1..20: mol_type = other DNA; note = GUSB primer forward sequence
tgcgtagggacaagaaccac

SEQ ID NO: 5 - DNA, 20 bp, synthetic construct
  source 1..20: mol_type = other DNA; note = GUSB primer reverse sequence
gggaggggtccaaggatttg

SEQ ID NO: 6 - DNA, 20 bp, synthetic construct
  source 1..20: mol_type = other DNA; note = IMMT primer forward sequence
aacccacacctgcactttca

SEQ ID NO: 7 - DNA, 20 bp, synthetic construct
  source 1..20: mol_type = other DNA; note = IMMT primer reverse sequence
ttttcctgttgtgcaaggcg

SEQ ID NO: 8 - DNA, 20 bp, synthetic construct
  source 1..20: mol_type = other DNA; note = EIF2S2 primer forward sequence
ccacaagtcgtccgagtagg

SEQ ID NO: 9 - DNA, 20 bp, synthetic construct
  source 1..20: mol_type = other DNA; note = EIF2S2 primer reverse sequence
ggagatgtttgggctgacga

SEQ ID NO: 10 - protein, 18 aa, synthetic construct
SESDDAMFCDAMDESDSK